European Patent Application EP 4 741 506 A1, published May 13, 2026. Title: 具有调节机体免疫能力的CpG寡聚脱氧核苷酸及其应用. Applicant: 南京吉盛澳玛生物医药有限公司. Application CN. The sequence listing filed with the application follows.

SEQUENCE LISTING (89 sequences)

SEQ ID NO: 1 - DNA, 21 bp, synthetic construct
  source 1..21: mol_type = other DNA
ggcgcgacgcgtcgcgggggg

SEQ ID NO: 2 - DNA, 22 bp, synthetic construct
  source 1..22: mol_type = other DNA
ggacgatcgagatcgtgggggg

SEQ ID NO: 3 - DNA, 20 bp, synthetic construct
  source 1..20: mol_type = other DNA
ggaggatcgatcctgggggg

SEQ ID NO: 4 - DNA, 22 bp, synthetic construct
  source 1..22: mol_type = other DNA
ggttcgatcgatcgaagggggg

SEQ ID NO: 5 - DNA, 22 bp, synthetic construct
  source 1..22: mol_type = other DNA
ggggcgatcgatcgaagggggg

SEQ ID NO: 6 - DNA, 22 bp, synthetic construct
  source 1..22: mol_type = other DNA
ggggcgatcgatcgaagggggg

SEQ ID NO: 7 - DNA, 22 bp, synthetic construct
  source 1..22: mol_type = other DNA
gggcgcgacgcgtcgcgggggg

SEQ ID NO: 8 - DNA, 21 bp, synthetic construct
  source 1..21: mol_type = other DNA
gggcgatcgatcgaagggggg

SEQ ID NO: 9 - DNA, 22 bp, synthetic construct
  source 1..22: mol_type = other DNA
ggggcgatcgatcgaagggggg

SEQ ID NO: 10 - DNA, 20 bp, synthetic construct
  source 1..20: mol_type = other DNA
ggcgatcgatcgaagggggg

SEQ ID NO: 11 - DNA, 19 bp, synthetic construct
  source 1..19: mol_type = other DNA
gcgatcgatcgaagggggg

SEQ ID NO: 12 - DNA, 16 bp, synthetic construct
  source 1..16: mol_type = other DNA
ggaggatcgatcctgg

SEQ ID NO: 13 - DNA, 18 bp, synthetic construct
  source 1..18: mol_type = other DNA
gggaggatcgatcctggg

SEQ ID NO: 14 - DNA, 20 bp, synthetic construct
  source 1..20: mol_type = other DNA
ggggaggatcgatcctgggg

SEQ ID NO: 15 - DNA, 22 bp, synthetic construct
  source 1..22: mol_type = other DNA
gggggaggatcgatcctggggg

SEQ ID NO: 16 - DNA, 24 bp, synthetic construct
  source 1..24: mol_type = other DNA
ggggggaggatcgatcctgggggg

SEQ ID NO: 17 - DNA, 26 bp, synthetic construct
  source 1..26: mol_type = other DNA
gggggggaggatcgatcctggggggg

SEQ ID NO: 18 - DNA, 28 bp, synthetic construct
  source 1..28: mol_type = other DNA
ggggggggaggatcgatcctgggggggg

SEQ ID NO: 19 - DNA, 30 bp, synthetic construct
  source 1..30: mol_type = other DNA
gggggggggaggatcgatcctggggggggg

SEQ ID NO: 20 - DNA, 32 bp, synthetic construct
  source 1..32: mol_type = other DNA
ggggggggggaggatcgatcctgggggggggg

SEQ ID NO: 21 - DNA, 34 bp, synthetic construct
  source 1..34: mol_type = other DNA
gggggggggggaggatcgatcctggggggggggg

SEQ ID NO: 22 - DNA, 22 bp, synthetic construct
  source 1..22: mol_type = other DNA
ggggaggatcgatcctgggggg

SEQ ID NO: 23 - DNA, 24 bp, synthetic construct
  source 1..24: mol_type = other DNA
ggggggaggatcgatcctgggggg

SEQ ID NO: 24 - DNA, 16 bp, synthetic construct
  source 1..16: mol_type = other DNA
ggcgatcgatcgaagg

SEQ ID NO: 25 - DNA, 18 bp, synthetic construct
  source 1..18: mol_type = other DNA
gggcgatcgatcgaaggg

SEQ ID NO: 26 - DNA, 20 bp, synthetic construct
  source 1..20: mol_type = other DNA
ggggcgatcgatcgaagggg

SEQ ID NO: 27 - DNA, 22 bp, synthetic construct
  source 1..22: mol_type = other DNA
gggggcgatcgatcgaaggggg

SEQ ID NO: 28 - DNA, 24 bp, synthetic construct
  source 1..24: mol_type = other DNA
ggggggcgatcgatcgaagggggg

SEQ ID NO: 29 - DNA, 26 bp, synthetic construct
  source 1..26: mol_type = other DNA
gggggggcgatcgatcgaaggggggg

SEQ ID NO: 30 - DNA, 28 bp, synthetic construct
  source 1..28: mol_type = other DNA
ggggggggcgatcgatcgaagggggggg

SEQ ID NO: 31 - DNA, 30 bp, synthetic construct
  source 1..30: mol_type = other DNA
gggggggggcgatcgatcgaaggggggggg

SEQ ID NO: 32 - DNA, 32 bp, synthetic construct
  source 1..32: mol_type = other DNA
ggggggggggcgatcgatcgaagggggggggg

SEQ ID NO: 33 - DNA, 34 bp, synthetic construct
  source 1..34: mol_type = other DNA
gggggggggggcgatcgatcgaaggggggggggg

SEQ ID NO: 34 - DNA, 23 bp, synthetic construct
  source 1..23: mol_type = other DNA
ggggcgatcgatcgaaagggggg

SEQ ID NO: 35 - DNA, 24 bp, synthetic construct
  source 1..24: mol_type = other DNA
ggggcgatcgatcgaaaagggggg

SEQ ID NO: 36 - DNA, 25 bp, synthetic construct
  source 1..25: mol_type = other DNA
ggggcgatcgatcgaaaaagggggg

SEQ ID NO: 37 - DNA, 24 bp, synthetic construct
  source 1..24: mol_type = other DNA
ggggggcgatcgatcgaagggggg

SEQ ID NO: 38 - DNA, 23 bp, synthetic construct
  source 1..23: mol_type = other DNA
gggggcgatcgatcgaagggggg

SEQ ID NO: 39 - DNA, 21 bp, synthetic construct
  source 1..21: mol_type = other DNA
gggcgatcgatcgaagggggg

SEQ ID NO: 40 - DNA, 20 bp, synthetic construct
  source 1..20: mol_type = other DNA
ggcgatcgatcgaagggggg

SEQ ID NO: 41 - DNA, 19 bp, synthetic construct
  source 1..19: mol_type = other DNA
gcgatcgatcgaagggggg

SEQ ID NO: 42 - DNA, 30 bp, synthetic construct
  source 1..30: mol_type = other DNA
ggggcgatcgatcgaaaaaaaaaagggggg

SEQ ID NO: 43 - DNA, 22 bp, synthetic construct
  source 1..22: mol_type = other DNA
ggggcgatcgatcgttgggggg

SEQ ID NO: 44 - DNA, 25 bp, synthetic construct
  source 1..25: mol_type = other DNA
ggggcgatcgatcgtttttgggggg

SEQ ID NO: 45 - DNA, 30 bp, synthetic construct
  source 1..30: mol_type = other DNA
ggggcgatcgatcgttttttttttgggggg

SEQ ID NO: 46 - DNA, 22 bp, synthetic construct
  source 1..22: mol_type = other DNA
ggggcgatcgatcgccgggggg

SEQ ID NO: 47 - DNA, 25 bp, synthetic construct
  source 1..25: mol_type = other DNA
ggggcgatcgatcgcccccgggggg

SEQ ID NO: 48 - DNA, 30 bp, synthetic construct
  source 1..30: mol_type = other DNA
ggggcgatcgatcgccccccccccgggggg

SEQ ID NO: 49 - DNA, 21 bp, synthetic construct
  source 1..21: mol_type = other DNA
ggggcgatcgatcgagggggg

SEQ ID NO: 50 - DNA, 20 bp, synthetic construct
  source 1..20: mol_type = other DNA
ggggcgatcgatcggggggg

SEQ ID NO: 51 - DNA, 19 bp, synthetic construct
  source 1..19: mol_type = other DNA
ggggacgatcgtcgggggg

SEQ ID NO: 52 - DNA, 18 bp, synthetic construct
  source 1..18: mol_type = other DNA
gggacgatcgtcgggggg

SEQ ID NO: 53 - DNA, 17 bp, synthetic construct
  source 1..17: mol_type = other DNA
ggacgatcgtcgggggg

SEQ ID NO: 54 - DNA, 16 bp, synthetic construct
  source 1..16: mol_type = other DNA
gacgatcgtcgggggg

SEQ ID NO: 55 - DNA, 21 bp, synthetic construct
  source 1..21: mol_type = other DNA
gggggacgatcgtcagggggg

SEQ ID NO: 56 - DNA, 22 bp, synthetic construct
  source 1..22: mol_type = other DNA
gggggacgatcgtcaagggggg

SEQ ID NO: 57 - DNA, 23 bp, synthetic construct
  source 1..23: mol_type = other DNA
gggggacgatcgtcaaagggggg

SEQ ID NO: 58 - DNA, 24 bp, synthetic construct
  source 1..24: mol_type = other DNA
gggggacgatcgtcaaaagggggg

SEQ ID NO: 59 - DNA, 25 bp, synthetic construct
  source 1..25: mol_type = other DNA
gggggacgatcgtcaaaaagggggg

SEQ ID NO: 60 - DNA, 30 bp, synthetic construct
  source 1..30: mol_type = other DNA
gggggacgatcgtcaaaaaaaaaagggggg

SEQ ID NO: 61 - DNA, 22 bp, synthetic construct
  source 1..22: mol_type = other DNA
gggggacgatcgtcttgggggg

SEQ ID NO: 62 - DNA, 25 bp, synthetic construct
  source 1..25: mol_type = other DNA
gggggacgatcgtctttttgggggg

SEQ ID NO: 63 - DNA, 30 bp, synthetic construct
  source 1..30: mol_type = other DNA
gggggacgatcgtcttttttttttgggggg

SEQ ID NO: 64 - DNA, 22 bp, synthetic construct
  source 1..22: mol_type = other DNA
gggggacgatcgtcccgggggg

SEQ ID NO: 65 - DNA, 25 bp, synthetic construct
  source 1..25: mol_type = other DNA
gggggacgatcgtccccccgggggg

SEQ ID NO: 66 - DNA, 30 bp, synthetic construct
  source 1..30: mol_type = other DNA
gggggacgatcgtcccccccccccgggggg

SEQ ID NO: 67 - DNA, 19 bp, synthetic construct
  source 1..19: mol_type = other DNA
gtgcatcgatgcagggggg

SEQ ID NO: 68 - DNA, 21 bp, synthetic construct
  source 1..21: mol_type = other DNA
gggtgcatcgatgcagggggg

SEQ ID NO: 69 - DNA, 22 bp, synthetic construct
  source 1..22: mol_type = other DNA
ggggtgcatcgatgcagggggg

SEQ ID NO: 70 - DNA, 23 bp, synthetic construct
  source 1..23: mol_type = other DNA
gggggtgcatcgatgcagggggg

SEQ ID NO: 71 - DNA, 21 bp, synthetic construct
  source 1..21: mol_type = other DNA
ggtgcatcgatgcaagggggg

SEQ ID NO: 72 - DNA, 22 bp, synthetic construct
  source 1..22: mol_type = other DNA
ggtgcatcgatgcaaagggggg

SEQ ID NO: 73 - DNA, 23 bp, synthetic construct
  source 1..23: mol_type = other DNA
ggtgcatcgatgcaaaagggggg

SEQ ID NO: 74 - DNA, 24 bp, synthetic construct
  source 1..24: mol_type = other DNA
ggtgcatcgatgcaaaaagggggg

SEQ ID NO: 75 - DNA, 25 bp, synthetic construct
  source 1..25: mol_type = other DNA
ggtgcatcgatgcaaaaaagggggg

SEQ ID NO: 76 - DNA, 30 bp, synthetic construct
  source 1..30: mol_type = other DNA
ggtgcatcgatgcaaaaaaaaaaagggggg

SEQ ID NO: 77 - DNA, 22 bp, synthetic construct
  source 1..22: mol_type = other DNA
ggtgcatcgatgcattgggggg

SEQ ID NO: 78 - DNA, 25 bp, synthetic construct
  source 1..25: mol_type = other DNA
ggtgcatcgatgcatttttgggggg

SEQ ID NO: 79 - DNA, 30 bp, synthetic construct
  source 1..30: mol_type = other DNA
ggtgcatcgatgcattttttttttgggggg

SEQ ID NO: 80 - DNA, 22 bp, synthetic construct
  source 1..22: mol_type = other DNA
ggtgcatcgatgcaccgggggg

SEQ ID NO: 81 - DNA, 25 bp, synthetic construct
  source 1..25: mol_type = other DNA
ggtgcatcgatgcacccccgggggg

SEQ ID NO: 82 - DNA, 30 bp, synthetic construct
  source 1..30: mol_type = other DNA
ggtgcatcgatgcaccccccccccgggggg

SEQ ID NO: 83 - DNA, 23 bp, synthetic construct
  source 1..23: mol_type = other DNA
ggggcgcgacgcgtcgcgggggg

SEQ ID NO: 84 - DNA, 20 bp, synthetic construct
  source 1..20: mol_type = other DNA
gggggacgatcgtcgggggg

SEQ ID NO: 85 - DNA, 20 bp, synthetic construct
  source 1..20: mol_type = other DNA
ggtgcatcgatgcagggggg

SEQ ID NO: 86 - DNA, 22 bp, synthetic construct
  source 1..22: mol_type = other DNA
tgactgtgaacgttcgagatga

SEQ ID NO: 87 - DNA, 22 bp, synthetic construct
  source 1..22: mol_type = other DNA
ggtgcgatcgatcgcagggggg

SEQ ID NO: 88 - DNA, 22 bp, synthetic construct
  source 1..22: mol_type = other DNA
ggtgcgatcgatcgcagggggg

SEQ ID NO: 89 - DNA, 22 bp, synthetic construct
  source 1..22: mol_type = other DNA
ggtgcgatcgatcgcagggggg